European Patent Application EP 4 527 458 A2, published March 26, 2025. Title: DPP3 binder directed to and binding to specific DPP3-epitopes and its use in the prevention or treatment of diseases / acute conditions that are associated with oxidative stress. Applicant: 4Teen4 Pharmaceuticals GmbH. Application EP, filed October 24, 2018. The sequence listing filed with the application follows.

SEQUENCE LISTING (30 sequences)

SEQ ID NO: 1 - protein, 737 aa, Homo sapiens
MADTQYILPNDIGVSSLDCREAFRLLSPTERLYAYHLSRAAWYGGLAVLLQTSPEAPYIYALLSRLFRAQDPDQLRQHALAEGLTEEEYQAFLVYAAGVYSNMGNYKSFGDTKFVPNLPKEKLERVILGSEAAQQHPEEVRGLWQTCGELMFSLEPRLRHLGLGKEGITTYFSGNCTMEDAKLAQDFLDSQNLSAYNTRLFKEVDGEGKPYYEVRLASVLGSEPSLDSEVTSKLKSYEFRGSPFQVTRGDYAPILQKVVEQLEKAKAYAANSHQGQMLAQYIESFTQGSIEAHKRGSRFWIQDKGPIVESYIGFIESYRDPFGSRGEFEGFVAVVNKAMSAKFERLVASAEQLLKELPWPPTFEKDKFLTPDFTSLDVLTFAGSGIPAGINIPNYDDLRQTEGFKNVSLGNVLAVAYATQREKLTFLEEDDKDLYILWKGPSFDVQVGLHELLGHGSGKLFVQDEKGAFNFDQETVINPETGEQIQSWYRSGETWDSKFSTIASSYEECRAESVGLYLCLHPQVLEIFGFEGADAEDVIYVNWLNMVRAGLLALEFYTPEAFNWRQAHMQARFVILRVLLEAGEGLVTITPTTGSDGRPDARVRLDRSKIRSVGKPALERFLRRLQVLKSTGDVAGGRALYEGYATVTDAPPECFLTLRDTVLLRKESRKLIVQPNTRLEGSDVQLLEYEASAAGLIRSFSERFPEDGPELEEILTQLATADARFWKGPSEAPSGQA

SEQ ID NO: 2 - protein, 21 aa, synthetic construct
CETVINPETGEQIQSWYRSGE

SEQ ID NO: 3 - protein, 6 aa, Homo sapiens
INPETG

SEQ ID NO: 4 - protein, 4 aa, Homo sapiens
ETGE

SEQ ID NO: 5 - protein, 116 aa, Synthetic construct
QVTLKESGPGILQPSQTLSLTCSFSGFSLSTSGMSVGWIRQPSGKGLEWLAHIWWNDNKSYNPALKSRLTISRDTSNNQVFLKIASVVTADTGTYFCARNYSYDYWGQGTTLTVSS

SEQ ID NO: 6 - protein, 112 aa, Synthetic construct
DVVVTQTPLSLSVSLGDPASISCRSSRSLVHSIGSTYLHWYLQKPGQSPKLLIYKVSNRFSGVPDRFSGSGSGTDFTLKISRVEAEDLGVYFCSQSTHVPWTFGGGTKLEIK

SEQ ID NO: 7 - protein, 10 aa, Synthetic construct
GFSLSTSGMS

SEQ ID NO: 8 - protein, 7 aa, Synthetic construct
IWWNDNK

SEQ ID NO: 9 - protein, 8 aa, Synthetic construct
ARNYSYDY

SEQ ID NO: 10 - protein, 11 aa, Synthetic construct
RSLVHSIGSTY

SEQ ID NO: 11 - protein, 9 aa, Synthetic construct
SQSTHVPWT

SEQ ID NO: 12 - protein, 469 aa, Synthetic construct
MDPKGSLSWRILLFLSLAFELSYGQITLKESGPTLVKPTQTLTLTCTFSGFSLSTSGMSVGWIRQPPGKALEWLAHIWWNDNKSYNPALKSRLTITRDTSKNQVVLTMTNMDPVDTGTYYCARNYSYDYWGQGTLVTVSSASTKGPSVFPLAPSSKSTSGGTAALGCLVKDYFPEPVTVSWNSGALTSGVHTFPAVLQSSGLYSLSSVVTVPSSSLGTQTYICNVNHKPSNTKVDKKVEPKSCDKTHTCPPCPAPELLGGPSVFLFPPKPKDTLMISRTPEVTCVVVDVSHEDPEVKFNWYVDGVEVHNAKTKPREEQYNSTYRVVSVLTVLHQDWLNGKEYKCKVSNKALPAPIEKTISKAKGQPREPQVYTLPPSRDELTKNQVSLTCLVKGFYPSDIAVEWESNGQPENNYKTTPPVLDSDGSFFLYSKLTVDKSRWQQGNVFSCSVMHEALHNHYTQKSLSLSPG

SEQ ID NO: 13 - protein, 239 aa, Synthetic construct
METDTLLLWVLLLWVPGSTGDIVMTQTPLSLSVTPGQPASISCKSSRSLVHSIGSTYLYWYLQKPGQSPQLLIYKVSNRFSGVPDRFSGSGSGTDFTLKISRVEAEDVGVYYCSQSTHVPWTFGGGTKVEIKRTVAAPSVFIFPPSDEQLKSGTASVVCLLNNFYPREAKVQWKVDNALQSGNSQESVTEQDSKDSTYSLSSTLTLSKADYEKHKVYACEVTHQGLSSPVTKSFNRGEC

SEQ ID NO: 14 - protein, 24 aa, Synthetic construct
  MOD_RES 1: note = N-terminal biotinylation
AFNFDQETVINPETGEQIQSWYRS

SEQ ID NO: 15 - protein, 19 aa, Synthetic construct
  MOD_RES 1: note = N-terminal biotinylation
AFNFDQETVINPETGEQIQ

SEQ ID NO: 16 - protein, 18 aa, Synthetic construct
  MOD_RES 1: note = N-terminal biotinylation
AFNFDQETVINPETGEQI

SEQ ID NO: 17 - protein, 17 aa, Synthetic construct
  MOD_RES 1: note = N-terminal biotinylation
AFNFDQETVINPETGEQ

SEQ ID NO: 18 - protein, 16 aa, Synthetic construct
  MOD_RES 1: note = N-terminal biotinylation
AFNFDQETVINPETGE

SEQ ID NO: 19 - protein, 15 aa, Synthetic construct
  MOD_RES 1: note = N-terminal biotinylation
AFNFDQETVINPETG

SEQ ID NO: 20 - protein, 14 aa, Synthetic construct
  MOD_RES 1: note = N-terminal biotinylation
AFNFDQETVINPET

SEQ ID NO: 21 - protein, 13 aa, Synthetic construct
  MOD_RES 1: note = N-terminal biotinylation
AFNFDQETVINPE

SEQ ID NO: 22 - protein, 12 aa, Synthetic construct
  MOD_RES 1: note = N-terminal biotinylation
AFNFDQETVINP

SEQ ID NO: 23 - protein, 11 aa, Synthetic construct
  MOD_RES 1: note = N-terminal biotinylation
AFNFDQETVIN

SEQ ID NO: 24 - protein, 11 aa, Synthetic construct
  MOD_RES 11: note = C-terminal biotinylation
ETGEQIQSWYK

SEQ ID NO: 25 - protein, 12 aa, Synthetic construct
  MOD_RES 12: note = C-terminal biotinylation
PETGEQIQSWYK

SEQ ID NO: 26 - protein, 13 aa, Synthetic construct
  MOD_RES 13: note = C-terminal biotinylation
NPETGEQIQSWYK

SEQ ID NO: 27 - protein, 14 aa, Synthetic construct
  MOD_RES 14: note = C-terminal biotinylation
INPETGEQIQSWYK

SEQ ID NO: 28 - protein, 15 aa, Synthetic construct
  MOD_RES 15: note = C-terminal biotinylation
VINPETGEQIQSWYK

SEQ ID NO: 29 - protein, 16 aa, Synthetic construct
  MOD_RES 16: note = C-terminal biotinylation
TVINPETGEQIQSWYK

SEQ ID NO: 30 - protein, 17 aa, Synthetic construct
  MOD_RES 17: note = C-terminal biotinylation
ETVINPETGEQIQSWYK